European Patent Application EP 4 446 438 A1, published October 16, 2024. Title: TAGGED LOOP PRIMER COMPRISING SINGLE-STRANDED INTERACTIVE DUAL LABELING SYSTEM AND NUCLEIC ACID ISOTHERMAL AMPLIFICATION METHOD USING THE SAME. Applicant: SEEGENE, INC. Application KR. The sequence listing filed with the application follows.

SEQUENCE LISTING (21 sequences)

SEQ ID NO: 1 - DNA, 21 bp, synthetic construct
  source 1..21: mol_type = other DNA
actgacttaacaaagccttac

SEQ ID NO: 2 - DNA, 25 bp, synthetic construct
  source 1..25: mol_type = other DNA
caccatcaacaaatatttttctcac

SEQ ID NO: 3 - DNA, 49 bp, synthetic construct
  source 1..49: mol_type = other DNA
tgggtggtatgtctgatcccaatagggatttgttaaaatatgacttcac

SEQ ID NO: 4 - DNA, 44 bp, synthetic construct
  source 1..44: mol_type = other DNA
tgtgttaactgtttggatgacagaggtccaaaacttgtaggtgg

SEQ ID NO: 5 - DNA, 24 bp, synthetic construct
  source 1..24: mol_type = other DNA
acggtcaaagagttttaacctctc

SEQ ID NO: 6 - DNA, 21 bp, synthetic construct
  source 1..21: mol_type = other DNA
tgcattctgcattgtgcaaac

SEQ ID NO: 7 - DNA, 59 bp, synthetic construct
  source 1..59: mol_type = other DNA
  misc_feature <1: function = CalRed610
  misc_feature 21..22: function = BHQ-2
ctcgcgaacgtatgctgtgctcctcgtggataggcacggtcaaagagttttaacctctc

SEQ ID NO: 8 - DNA, 18 bp, synthetic construct
  source 1..18: mol_type = other DNA
caagctttcggcagacgt

SEQ ID NO: 9 - DNA, 25 bp, synthetic construct
  source 1..25: mol_type = other DNA
ggatctttgtcatccaatttgatgg

SEQ ID NO: 10 - DNA, 47 bp, synthetic construct
  source 1..47: mol_type = other DNA
tgcggccaatgtttgtaatcagttctccagaacaaacccaaggaaat

SEQ ID NO: 11 - DNA, 40 bp, synthetic construct
  source 1..40: mol_type = other DNA
ccagcgcttcagcgttcttcgacctgtgtaggtcaaccac

SEQ ID NO: 12 - DNA, 25 bp, synthetic construct
  source 1..25: mol_type = other DNA
tgtctgattagttcctggtccccaa

SEQ ID NO: 13 - DNA, 20 bp, synthetic construct
  source 1..20: mol_type = other DNA
tcgcgcattggcatggaagt

SEQ ID NO: 14 - DNA, 55 bp, synthetic construct
  source 1..55: mol_type = other DNA
  misc_feature <1: function = Quasar670
  misc_feature 21..22: function = BHQ-2
cgacggatgcaacgtagcgatcatgcaacgtacgctcgcgcattggcatggaagt

SEQ ID NO: 15 - DNA, 18 bp, synthetic construct
  source 1..18: mol_type = other DNA
ttcaagggcccggctcta

SEQ ID NO: 16 - DNA, 25 bp, synthetic construct
  source 1..25: mol_type = other DNA
ggcactggaaattgtataccttctc

SEQ ID NO: 17 - DNA, 50 bp, synthetic construct
  source 1..50: mol_type = other DNA
acagttatgcagactaaatccacattgttgttgcagtttttccaaagaca

SEQ ID NO: 18 - DNA, 47 bp, synthetic construct
  source 1..47: mol_type = other DNA
accattttacttcaaaagacctcctagcagggctatagacaagttca

SEQ ID NO: 19 - DNA, 25 bp, synthetic construct
  source 1..25: mol_type = other DNA
tgtgtgcaagcaatatgaaaaagct

SEQ ID NO: 20 - DNA, 18 bp, synthetic construct
  source 1..18: mol_type = other DNA
ttgaccgaggcctggctt

SEQ ID NO: 21 - DNA, 53 bp, synthetic construct
  source 1..53: mol_type = other DNA
  misc_feature <1: function = CalOrange560
  misc_feature 21..22: function = BHQ-2
agtcgaccgtactgtcgtactcgtcgcgcgaacgtttgaccgaggcctggctt